European Patent Application EP 4 273 169 A1, published November 8, 2023. Title: DEVELOPMENT AND USE OF FUNCTION-ENHANCED ANTIBODY BLOCKING AGENT. Applicant: Keymed Biosciences Co.,Ltd. The sequence listing filed with the application follows.

SEQUENCE LISTING (162 sequences)

SEQ ID NO: 1 - protein, 702 aa, Artificial Sequence
  synthetically generated protein
ESLGWDVAELQLNHTGPQQDPRLYWQGGPALGRSFLHGPELDKGQLRIHRDGIYMVHIQVTLAICSSTTASRHHPTTLAVGICSPASRSISLLRLSFHQGCTIASQRLTPLARGDTLCTNLTGTLLPSRNTDETFFGVQWVRPGSGSGNGSESLGWDVAELQLNHTGPQQDPRLYWQGGPALGRSFLHGPELDKGQLRIHRDGIYMVHIQVTLAICSSTTASRHHPTTLAVGICSPASRSISLLRLSFHQGCTIASQRLTPLARGDTLCTNLTGTLLPSRNTDETFFGVQWVRPGSGSGNGSESLGWDVAELQLNHTGPQQDPRLYWQGGPALGRSFLHGPELDKGQLRIHRDGIYMVHIQVTLAICSSTTASRHHPTTLAVGICSPASRSISLLRLSFHQGCTIASQRLTPLARGDTLCTNLTGTLLPSRNTDETFFGVQWVRPASGGGGSEPRGPTIKPCPPCKCPAPNLLGGPSVFIFPPKIKDVLMISLSPIVTCVVVDVSEDDPDVQISWFVNNVEVHTAQTQTHREDYNSTLRVVSALPIQHQDWMSGKEFKCKVNNKDLPAPIERTISKPKGSVRAPQVYVLPPCEEEMTKKQVTLWCMVTDFMPEDIYVEWTNNGKTELNYKNTEPVLDSDGSYFMYSKLRVEKKNWVERNSYSCSVVHEGLHNHHTTKSFSRTPGKGSGLNDIFEAQKIEWHE

SEQ ID NO: 2 - protein, 240 aa, Mus musculus
ASGGGGSEPRGPTIKPCPPCKCPAPNLLGGPSVFIFPPKIKDVLMISLSPIVTCVVVDVSEDDPDVQISWFVNNVEVHTAQTQTHREDYNSTLRVVSALPIQHQDWMSGKEFKCKVNNKDLPAPIERTISKPKGSVRAPQVCVLPPPEEEMTKKQVTLSCAVTDFMPEDIYVEWTNNGKTELNYKNTEPVLDSDGSYFMVSKLRVEKKNWVERNSYSCSVVHEGLHNHHTTKSFSRTPGK

SEQ ID NO: 3 - protein, 120 aa, Mus musculus
QVQLQQSGPGLVQPSQSLSITCTVSGFSLTTYAVHWVRQSPGKGLEWLGVIWSTGITDYNAAFISRLSISKDNSKSQVFFKMNSLQSDDIAIYYCARNPYYGNLNAMDYWGQGTSVTVSS

SEQ ID NO: 4 - DNA, 360 bp, Mus musculus
caggtgcagctgcagcagtcaggacctggcctagtgcagccctcacagagcctgtccatcacctgcacagtctctggtttctcattaactacctatgctgtgcactgggttcgccagtctccaggaaagggtctggagtggctgggagtgatatggagtactggaatcacagactataatgcagctttcatatccagactgagcatcagcaaggacaactccaagagccaagttttctttaaaatgaacagtctgcaatctgatgacatagccatatactactgtgccagaaatccctactatggtaacctcaatgctatggactactggggtcaaggaacctcagtcaccgtctcctca

SEQ ID NO: 5 - protein, 9 aa, Mus musculus
FSLTTYAVH

SEQ ID NO: 6 - protein, 16 aa, Mus musculus
VIWSTGITDYNAAFIS

SEQ ID NO: 7 - protein, 12 aa, Mus musculus
NPYYGNLNAMDY

SEQ ID NO: 8 - protein, 111 aa, Mus musculus
DIVLTQSPASLAVSLGQRATISCRASKSVDTSGYSFMHWYQQKPGQPPKLLIYLASNLESGVPARFSGSGSGTDFTLNIHPVEEEDAATYYCQHSRELPLTFGAGTKLELK

SEQ ID NO: 9 - DNA, 333 bp, Mus musculus
gacattgtgctgacacagtctcctgcttccttagctgtatctctggggcagagggccaccatctcatgcagggccagcaaaagtgtcgatacatctggctatagttttatgcactggtaccaacagaaaccaggacagccacccaaactcctcatctatcttgcatccaacctagaatctggggtccctgccaggttcagtggcagtgggtctgggacagacttcaccctcaacatccatcctgtggaggaggaggatgctgcaacctattactgtcagcacagtagggagcttcctctcacgttcggtgctgggaccaagctggagctgaaa

SEQ ID NO: 10 - protein, 15 aa, Mus musculus
RASKSVDTSGYSFMH

SEQ ID NO: 11 - protein, 7 aa, Mus musculus
LASNLES

SEQ ID NO: 12 - protein, 9 aa, Mus musculus
QHSRELPLT

SEQ ID NO: 13 - protein, 120 aa, Mus musculus
EVQLKQSGPGLVQPSQSLSITCTVSGFSLTTYGVHWVRQSPGKGLEWLGVIWSTGITDYNAAFISRLSISKDNSKSQVFFKMNSLQADDTAIYYCARNSYYGNLYVMDYWGQGTSVTVSS

SEQ ID NO: 14 - DNA, 360 bp, Mus musculus
gaggtgcagctgaagcagtcaggacctggcctagtgcagccctcacagagcctgtccatcacctgcacagtctctggtttttcattaactacctatggtgtacactgggttcgccagtctccaggaaagggtctggagtggctgggagtgatatggagtactggaatcacagactataatgcagctttcatatccagactgagcatcagtaaggacaattccaagagccaagtcttctttaaaatgaacagtctgcaagctgatgacacagccatatattactgtgccagaaattcctactatggtaacctttatgttatggactactggggtcaaggaacctcagtcaccgtctcctca

SEQ ID NO: 15 - protein, 9 aa, Mus musculus
FSLTTYGVH

SEQ ID NO: 16 - protein, 12 aa, Mus musculus
NSYYGNLYVMDY

SEQ ID NO: 17 - protein, 111 aa, Mus musculus
DIVLTQSPASLAVSLGQRATISCRASKSVSASGYNFMHWYQQKPGQPPKLLIYLASNLESGVPARFSGSGSGTDFTLNIHPVEEEDAATYYCQHSRELPLTFGAGTKLELK

SEQ ID NO: 18 - DNA, 333 bp, Mus musculus
gacattgtgctaacacagtctcctgcttccttagctgtgtctctggggcagagggccaccatctcatgcagggccagcaaaagtgtcagtgcatctggctataattttatgcactggtatcaacagaaaccaggacagccacccaaactcctcatctatcttgcatccaacctagaatctggggtccctgccaggttcagtggcagtgggtctgggacagacttcaccctcaacatccatcctgtggaggaggaggatgctgcaacctattactgtcagcacagtagggagcttccgctcacgttcggtgctgggaccaagctggagctgaaa

SEQ ID NO: 19 - protein, 15 aa, Mus musculus
RASKSVSASGYNFMH

SEQ ID NO: 20 - protein, 120 aa, Mus musculus
QVQLQQSGPGLVQPSQSLSITCTVSGFSLTTYAVHWVRQSPGKGLEWLGVIWSTGITDYNAAFISRLSISKDNSKSQVFFKMDSLQSDDTAIYFCARNPHYGNLNAMDYWGQGTSVTVSS

SEQ ID NO: 21 - DNA, 360 bp, Mus musculus
caggtgcagctgcagcagtcaggacctggcctagtgcagccctcacagagcctgtccatcacctgcacagtctctggtttctcattaactacctatgctgtgcactgggttcgccagtctccaggaaagggtctggagtggctgggagtaatatggagtactggaatcacagactataatgcagctttcatatccagactgagcatcagcaaggacaactccaagagccaagttttctttaaaatggacagtctgcaatctgatgacacagccatatacttctgtgccagaaatccccactatggtaatctcaatgctatggactactggggtcaaggaacctcagtcaccgtctcctca

SEQ ID NO: 22 - protein, 12 aa, Mus musculus
NPHYGNLNAMDY

SEQ ID NO: 23 - protein, 111 aa, Mus musculus
DIVLTQSPASLAVSLGQRATISCRASKSVSASGYTWMHWYQQKPGQAPKLLIYLASNLESGVPARFSGSGSGTDFTLNIHPVEEEDAATYYCQHSRELPPTFGGGTKLEIK

SEQ ID NO: 24 - DNA, 333 bp, Mus musculus
gacattgtgctgacacagtctcctgcttccttagctgtatctctggggcagagggccaccatctcatgcagggccagcaaaagcgtcagtgcatctggctatacttggatgcactggtaccaacagaaaccaggacaggcacccaaactcctcatctatcttgcatccaacctagaatctggggtccctgccaggttcagtggcagtgggtctgggacagacttcaccctcaacatccatcctgtggaggaggaggatgctgcaacctattactgtcagcacagtagggagcttcctccgacgttcggtggaggcaccaagctggaaatcaaa

SEQ ID NO: 25 - protein, 15 aa, Mus musculus
RASKSVSASGYTWMH

SEQ ID NO: 26 - protein, 9 aa, Mus musculus
QHSRELPPT

SEQ ID NO: 27 - protein, 120 aa, Mus musculus
EVQLQQSGPELVKPGASVKMSCKASGYTFTDYVIHWVKQKPGQGLEWIGYLHPYNDDTKYNEKFKGKATLTSDKSSSTAYMELSSLTSEDSAVYYCARRGYYDYAWFADWGQGTLVTVSA

SEQ ID NO: 28 - DNA, 360 bp, Mus musculus
gaggtccagctgcagcagtctggacctgagctggtaaagcctggggcttcagtgaagatgtcctgcaaggcttctggatacacattcactgactatgttatacactgggtgaagcagaagcctgggcagggccttgagtggattggatatcttcatccttacaatgatgatactaagtacaatgagaagttcaaaggcaaggccacactgacttcagacaaatcctccagcacagcctacatggagctcagcagcctgacctctgaggactctgcggtctattactgtgcaagacgggggtactatgattacgcctggtttgctgactggggccaagggactctggtcactgtctctgca

SEQ ID NO: 29 - protein, 9 aa, Mus musculus
YTFTDYVIH

SEQ ID NO: 30 - protein, 17 aa, Mus musculus
YLHPYNDDTKYNEKFKG

SEQ ID NO: 31 - protein, 11 aa, Mus musculus
RGYYDYAWFAD

SEQ ID NO: 32 - protein, 111 aa, Mus musculus
DIVLTQSPASLAVSLGQRATISCRASKSVSASGYTWIHWYQQKPRQAPKLLIYLASNLESGVPARFSGSGSGTDFTLNIHPVEEEDAATYYCQHSRELPPTFGGGTKLEIK

SEQ ID NO: 33 - DNA, 333 bp, Mus musculus
gacattgtgctaacacagtctcctgcttccttagctgtatctctggggcagagggccaccatctcatgcagggccagcaaaagtgtcagtgcatctggctatacttggatacactggtaccaacagaaaccaagacaggcacccaaacttctcatctatcttgcatccaacctagaatctggggtccctgccaggttcagtggcagtgggtctgggacagacttcaccctcaacatccatcctgtggaggaggaggatgctgcaacctattactgtcagcacagtagggaacttcctccgacgttcggtggaggcaccaagctggaaatcaaa

SEQ ID NO: 34 - protein, 15 aa, Mus musculus
RASKSVSASGYTWIH

SEQ ID NO: 35 - protein, 120 aa, Mus musculus
QVQLQQSGPGLVQPSQSLSITCTVSGFSLTTYAVHWVRQSPGKGLEWLGVIWSVGSTDYNAAFISRLSISKDNSKSQVFFKMNSLQADDTAIYYCARNIYYGNVYAMDYWGQGTSVTVSS

SEQ ID NO: 36 - DNA, 360 bp, Mus musculus
caggtgcagctgcagcagtcaggacctggcctagtgcagccctcacagagcctgtccatcacctgcacagtctctggtttctcattaactacctatgctgtacactgggttcgccagtctccaggaaagggtctggagtggctgggagttatatggagtgttggaagcacagactataatgcagctttcatatccagactgagcatcagcaaggacaattccaagagccaagttttctttaaaatgaacagtctgcaagctgatgacacagccatatattactgtgccagaaatatctactatggtaatgtttatgctatggactactggggtcaaggaacctcagtcaccgtctcctca

SEQ ID NO: 37 - protein, 16 aa, Mus musculus
VIWSVGSTDYNAAFIS

SEQ ID NO: 38 - protein, 12 aa, Mus musculus
NIYYGNVYAMDY

SEQ ID NO: 39 - protein, 111 aa, Mus musculus
DIVLTQSPASLAVSLGQRATISCRASKSVDASGYSFMHWYQQKAGQPPKLLIYLASNLESGVPARFSGRGSGTDFTLNIHPVEEGDAATYYCQHSRELPLTFGAGTKLEIK

SEQ ID NO: 40 - DNA, 333 bp, Mus musculus
gacattgtgctaacacagtctcctgcttccttagctgtatctctggggcagagggccaccatctcatgcagggccagcaaaagtgtcgatgcatctggctatagttttatgcactggtaccaacagaaagcaggacagccacccaaactcctcatctatcttgcatccaacctagaatctggggtccctgccaggttcagtggcagggggtctgggacagacttcaccctcaacatccatcctgtggaggagggggatgctgcaacctattactgtcagcacagtagggagcttcctctcacgttcggggctgggaccaagctggaaatcaaa

SEQ ID NO: 41 - protein, 15 aa, Mus musculus
RASKSVDASGYSFMH

SEQ ID NO: 42 - protein, 119 aa, Mus musculus
EIQLVQSGPELKKPGETVKISCKASGYTFTNYGMNWVKQTPGKGLKWMGWINTDTGEPTYADDFKGRFAFSLETSASTAYLQINNLKNEDMATYFCAREEDYRYVFNYWGQGTTLTVSS

SEQ ID NO: 43 - DNA, 357 bp, Mus musculus
gagatccagctggtgcagtctggacctgagctgaagaagcctggagagactgtcaagatctcctgcaaggcttctggatataccttcacaaactatggaatgaactgggtgaagcagactccaggaaagggtttaaagtggatgggctggataaacaccgacactggagagccaacatatgctgatgacttcaagggacggtttgccttctctttggaaacctctgccagcactgcctatttgcagatcaacaacctcaaaaatgaggacatggctacatatttctgtgcaagagaggaggactataggtacgtttttaattactggggccaaggcaccactctcacagtctcctca

SEQ ID NO: 44 - protein, 9 aa, Mus musculus
YTFTNYGMN

SEQ ID NO: 45 - protein, 17 aa, Mus musculus
WINTDTGEPTYADDFKG

SEQ ID NO: 46 - protein, 10 aa, Mus musculus
EEDYRYVFNY

SEQ ID NO: 47 - protein, 107 aa, Mus musculus
DIQMTQTTSSLSASLGDRVTISCRASQDISNYLNWYQQKPDGTVKLLIYYTSRLHSGVPSRFSGSGSGTDYSLTISNLEQEDIATYFCQQGVTLPLTFGAGTKLELK

SEQ ID NO: 48 - DNA, 321 bp, Mus musculus
gatatccagatgacacagactacatcctccctgtctgcctctctgggagacagagtcaccatcagttgcagggcaagtcaggacattagcaattatttaaactggtatcagcagaaaccagatggaactgttaaactcctgatctactacacatcaagattacactcaggagtcccatcaaggttcagtggcagtgggtctggaacagattattctctcaccattagcaacctggagcaagaagatattgccacttacttttgccaacagggtgttacgcttcctctcacgttcggtgctgggaccaagctggagctgaaa

SEQ ID NO: 49 - protein, 11 aa, Mus musculus
RASQDISNYLN

SEQ ID NO: 50 - protein, 7 aa, Mus musculus
YTSRLHS

SEQ ID NO: 51 - protein, 9 aa, Mus musculus
QQGVTLPLT

SEQ ID NO: 52 - protein, 121 aa, Mus musculus
QVQLQQSGPELVKPGASVKISCKTSGYTFADYTMHWVRQSQGKSLEWIGDIYPNDGGPNNNQKFKDKATLTVDKSSSTAYMELRSLTSEDSAVYYCARPFYYGNYAGFAFWGQGTLVTVSA

SEQ ID NO: 53 - DNA, 363 bp, Mus musculus
caggttcagctgcaacagtctggacctgagctggtgaagcctggggcttcagtgaagatatcctgcaagacttctggatacacattcgctgattacaccatgcactgggtgaggcagagccaaggaaagagccttgagtggattggagatatttatcctaacgatggtggtcctaacaacaaccagaagttcaaggacaaggccacattgactgttgacaagtcctccagcacagcctacatggagctccgcagcctgacatctgaggattctgcagtctattactgtgcaagaccgttctattatggtaactacgcgggatttgctttctggggccaagggactctggtcactgtctctgca

SEQ ID NO: 54 - protein, 9 aa, Mus musculus
YTFADYTMH

SEQ ID NO: 55 - protein, 17 aa, Mus musculus
DIYPNDGGPNNNQKFKD

SEQ ID NO: 56 - protein, 12 aa, Mus musculus
PFYYGNYAGFAF

SEQ ID NO: 57 - protein, 106 aa, Mus musculus
EMVLTQSPAIMSASPGEKVTMTCSASSSVSYMYWYQQKPGSSPRLLIYDTSNLASGVPVRFSGSGSGTSYSLTISRMEAEDAATYYCQQWSSYPLTFGAGTRLEIK

SEQ ID NO: 58 - DNA, 318 bp, Mus musculus
gaaatggttctcacccagtctccagcaatcatgtctgcatctccaggggagaaggtcaccatgacctgcagtgccagctcaagtgtaagttacatgtactggtaccagcagaagccaggatcctcccccagactcctgatttatgacacatccaacctggcttctggagtccctgttcgcttcagtggcagtgggtctgggacctcttactctctcacaatcagccgaatggaggctgaagatgctgccacttattactgccagcagtggagtagttacccgctcacgttcggtgctgggaccagactggaaataaaa

SEQ ID NO: 59 - protein, 10 aa, Mus musculus
SASSSVSYMY

SEQ ID NO: 60 - protein, 7 aa, Mus musculus
DTSNLAS

SEQ ID NO: 61 - protein, 9 aa, Mus musculus
QQWSSYPLT

SEQ ID NO: 62 - protein, 120 aa, Mus musculus
EVQLQESGPGLVQPSQSLSITCTVSGFSLTTYAVHWVRQSPGKGLEWLGVIWSTGITDYNADFISRLSISKDNSKSQVFFKMDSLQSDDTAIYFCARNHYYGNLNAMDYWGQGTSVTVSS

SEQ ID NO: 63 - DNA, 360 bp, Mus musculus
gaggtccagctgcaggagtcaggacctggcctagtgcagccctcacagagcctatccatcacctgcacagtctctggtttctcattaactacctatgctgtacactgggttcgccagtctccaggaaagggtctggagtggctgggagtaatatggagtactggaatcacagactataatgcagatttcatatccagactgagcatcagcaaggacaactccaagagccaagttttctttaaaatggacagtctgcaatctgatgacacagccatatacttctgtgccagaaatcactactatggcaatctcaatgctatggactactggggtcaaggaacctcagtcaccgtctcctca

SEQ ID NO: 64 - protein, 16 aa, Mus musculus
VIWSTGITDYNADFIS

SEQ ID NO: 65 - protein, 12 aa, Mus musculus
NHYYGNLNAMDY

SEQ ID NO: 66 - protein, 111 aa, Mus musculus
DIVLTQSPASLAVSLGQRATISCRASKSVSTSGYSFMHWYQQKPGQPPKLLIYLASNLESGVPARFSGSGSGTDFTLNIHPVEEEDAATYYCQHSRELPYTFGGGTKLEIK

SEQ ID NO: 67 - DNA, 333 bp, Mus musculus
gacattgtgctaacacagtctcctgcttccttagctgtatctctggggcagagggccaccatctcatgcagggccagcaaaagtgtcagtacatctggctatagttttatgcactggtaccaacagaaaccaggacagccacccaaactcctcatctatcttgcatccaacctagaatctggggtccctgccaggttcagtggcagtgggtctgggacagacttcaccctcaacatccatcctgtggaggaggaggatgctgcaacctattactgtcagcacagtagggagcttccgtacacgttcggaggggggaccaagctggaaatcaaa

SEQ ID NO: 68 - protein, 15 aa, Mus musculus
RASKSVSTSGYSFMH

SEQ ID NO: 69 - protein, 9 aa, Mus musculus
QHSRELPYT

SEQ ID NO: 70 - protein, 120 aa, Mus musculus
EVQLQQSGPELVKPGASLKMSCKASGYTFTDYVIHWVKQKPGQGLEWIGYLHPYNDDTKYNEKFKGKATLTSDKSSSTAYMELNSLTSEDSAVYYCARRGYYDYAWFADWGQGTLVTVSA

SEQ ID NO: 71 - DNA, 360 bp, Mus musculus
gaggtccagttgcagcagtctggacctgagctggtaaagcctggggcttcactgaagatgtcctgcaaggcttctggatacacattcactgactatgttatacactgggtgaagcagaagcctgggcagggccttgagtggattggatatcttcatccttacaatgatgatactaagtacaatgagaagttcaaaggcaaggccacactgacttcagacaaatcctccagcacagcctacatggaactcaacagcctgacctctgaggactctgcggtctattactgtgcaaggcgggggtactatgattacgcctggtttgctgactggggccaagggactctggtcactgtctctgca

SEQ ID NO: 72 - protein, 111 aa, Mus musculus
DIVLTQSPASLAVSLGQRATISCKASKSVSASGYTWMHWYQQKPGQAPKLLIYLASNLESGVPARFSGSGSGTDFTLNIHPVEEEDAATYYCQHSRELPPTFGGGTKLEIK

SEQ ID NO: 73 - DNA, 333 bp, Mus musculus
gacattgtgctaacacagtctcctgcttccttagctgtatctctggggcagagggccaccatctcatgcaaggccagcaaaagtgtcagtgcatctggctatacttggatgcactggtaccaacagaaaccaggacaggcacccaaactcctcatctatcttgcatccaacctagaatctggggtccctgccaggttcagtggcagtgggtctgggacagacttcaccctcaacatccatcctgtggaggaggaggatgctgcaacctattactgtcagcacagtagggagcttcctccgacgttcggtggaggcaccaagctggaaatcaaa

SEQ ID NO: 74 - protein, 15 aa, Mus musculus
KASKSVSASGYTWMH

SEQ ID NO: 75 - protein, 119 aa, Mus musculus
EIQLVQSGPELKKPGETVKISCKASGYTFTNYGMNWVKQAPGQGLKWMGWINTYTGEPTYADDFTGRFAFSLETSASTAYLQINNLKNEDMAAYFCAREEDYRYVFNYWGQGTTLTVSS

SEQ ID NO: 76 - DNA, 357 bp, Mus musculus
gagatccagttggtgcagtctggacctgagctgaagaagcctggagagacagtcaagatctcctgcaaggcttctgggtataccttcacaaactatggaatgaactgggtgaagcaggctccaggacagggtttaaagtggatgggctggataaacacctatactggagagccaacatatgctgatgacttcacgggacggtttgccttctccttggaaacctctgccagcactgcctatttgcagatcaacaacctcaaaaatgaggacatggctgcatatttctgtgcaagagaggaggactataggtacgtttttaactactggggccaaggcaccactctcacagtctcctca

SEQ ID NO: 77 - protein, 17 aa, Mus musculus
WINTYTGEPTYADDFTG

SEQ ID NO: 78 - protein, 107 aa, Mus musculus
DIQMIQSTSSLSASLGNRVTISCRASQDISNYLNWYQQKPDGTVKLLIYDTSRLHAGVPSRFSGSGSGTDYSLTISNLEQEDIATYFCQQGVTLPLTFGAGTKLEIK

SEQ ID NO: 79 - DNA, 321 bp, Mus musculus
gacatccagatgattcagtctacatcctccctgtctgcctctctgggaaacagagtcaccatcagttgcagggcaagtcaggacattagcaattatttaaactggtatcagcagaaaccagatggaactgttaaactcctgatctacgacacatcaagattacacgcaggagtcccatcaaggttcagtggcagtgggtctggaacagattattctctcaccattagcaacctggagcaagaagatatcgccacttacttttgccaacagggtgttacgcttcctctcacgttcggtgctgggaccaagctggaaataaaa

SEQ ID NO: 80 - protein, 7 aa, Mus musculus
DTSRLHA

SEQ ID NO: 81 - protein, 120 aa, Mus musculus
QVQLKQSGPGLVQPSQSLSITCTVSGFSLTSYGIHWVRQSPGKGLEWLGVIWSGGSTDFNAAFISRLSISKDNSKSQVFFKVISLQANDTAIYYCGRNSYYGNLYAMDYWGQGTSVTVSS

SEQ ID NO: 82 - DNA, 360 bp, Mus musculus
caggtccagctgaagcagtcaggacctggcctagtgcagccctcacagagcctgtccatcacctgcacagtctctggtttctcattaactagctatggtatacactgggttcgccagtctccaggaaagggtctggagtggctgggagtgatatggagtggtggaagcacagactttaatgcagctttcatatcaagactgagcatcagcaaggacaattccaagagccaagttttctttaaagtgatcagtctgcaagctaatgacacagccatatattactgtggcagaaattcctactatggtaatctctatgctatggactactggggtcaaggaacctcagtcaccgtctcctca

SEQ ID NO: 83 - protein, 9 aa, Mus musculus
FSLTSYGIH

SEQ ID NO: 84 - protein, 16 aa, Mus musculus
VIWSGGSTDFNAAFIS

SEQ ID NO: 85 - protein, 12 aa, Mus musculus
NSYYGNLYAMDY

SEQ ID NO: 86 - protein, 111 aa, Mus musculus
DIVLTQSPTSLAVSLGQRATISCRASKSVSASGYSFMHWYQQKPGQPPKLLIYLASNLESGVPARFSGSGSGTDFTLNIHPVEEEDAATYYCQHSRELPLTFGAGTKLELK

SEQ ID NO: 87 - DNA, 333 bp, Mus musculus
gacattgtgctgacacagtctcctacttccttagctgtatctctggggcagagggccaccatctcatgcagggccagcaaaagtgtcagtgcatctggctatagttttatgcactggtaccaacagaaaccaggacagccacccaaactcctcatctatcttgcatccaacctagaatctggggtccctgccaggttcagtggcagtgggtctgggacagacttcaccctcaacatccatcctgtggaggaggaggatgctgcaacctattactgtcagcacagtcgggagcttcctctcacgttcggtgctgggaccaagctggagctgaaa

SEQ ID NO: 88 - protein, 15 aa, Mus musculus
RASKSVSASGYSFMH

SEQ ID NO: 89 - protein, 120 aa, Mus musculus
QVQLQQSGPGLVQPSQSLSITCTVSGFSLTTYAVHWFRQSPGQGLEWLGVIWSTGITDFNAAFISRLNINKDSSKSQIFFKMISLQPNDTAIYYCGRNSYYGNLYAMDYWGQGTSVTVSS

SEQ ID NO: 90 - DNA, 360 bp, Mus musculus
caggtgcagctgcagcagtcaggacctggcctagtgcagccctcacagagcctgtccatcacctgcacagtctctggtttctcattaactacctatgctgttcactggtttcgccagtctccaggacagggtctggagtggctgggagtgatatggagtactggaatcacagactttaatgcagctttcatatcaagactgaacatcaacaaagacagttccaagagccagattttctttaaaatgatcagtctgcaacctaatgacacagccatatattactgtggcagaaattcctactatggtaatctctatgctatggactactggggtcaaggaacctcagtcaccgtctcctca

SEQ ID NO: 91 - protein, 16 aa, Mus musculus
VIWSTGITDFNAAFIS

SEQ ID NO: 92 - protein, 111 aa, Mus musculus
DIVLTQSPTSLAVSLGQRATISCRASKSVSASGYNFMHWYQQKPGQPPKLLIYLASNLESGVPARFSGSGSETDFTLNIHPVEEGDAATYYCQHSRELPLTFGAGTKLELK

SEQ ID NO: 93 - DNA, 333 bp, Mus musculus
gacattgtgctgacacagtctcctacttccttagctgtatctctggggcagagggccaccatctcatgcagggccagtaaaagtgtcagtgcatctggctataattttatgcactggtaccaacagaaaccaggtcagccacccaaactcctcatctatcttgcatccaacctagaatctggggtccctgccaggttcagtggcagtgggtctgagacagacttcaccctcaacatccatcctgtggaggagggggatgctgcaacctattactgtcaacacagtcgggagcttcctctcacgttcggtgctgggaccaagctggagctgaaa

SEQ ID NO: 94 - protein, 120 aa, Mus musculus
QVQLKQSGPGLVQPSQSLSITCTVSNFSLSTYGVHWVRQSPGKGLEWLGVIWGGGYTDYNAAFISRLTISKDNSKSQVFFKMNSLQADDTAIYYCARNNYYGNLYAMDYWGQGTSVTVSS

SEQ ID NO: 95 - DNA, 360 bp, Mus musculus
caggtccagctgaagcagtcaggacctggcctagtgcagccctcacagagcctgtccatcacctgcacagtctctaatttctcattaagtacctatggtgtacactgggttcgccagtctccaggaaagggtctggagtggctgggagtgatctggggtggtggatacacagactataatgcagctttcatatccagactgaccatcagcaaggacaactccaagagccaagttttctttaaaatgaacagtctgcaagctgatgacacagccatatattattgtgccagaaataactactatggtaacctctatgctatggactactggggtcaaggaacctcagtcaccgtctcctca

SEQ ID NO: 96 - protein, 9 aa, Mus musculus
FSLSTYGVH

SEQ ID NO: 97 - protein, 16 aa, Mus musculus
VIWGGGYTDYNAAFIS

SEQ ID NO: 98 - protein, 12 aa, Mus musculus
NNYYGNLYAMDY

SEQ ID NO: 99 - protein, 111 aa, Mus musculus
DIVLTQSPASLPVSLGQRATISCRANKSVSASGYSFMHWYQQKPGQPPKLLIYLASNLDSGVPARFSGSGSGTDFTLNIHPVEEEDTATYYCQHSREFPLTFGAGTKLELK

SEQ ID NO: 100 - DNA, 333 bp, Mus musculus
gacattgtgctgacacagtctcctgcttccttacctgtatctctggggcagagggccaccatctcatgcagggccaacaaaagtgtcagtgcatctggctatagttttatgcactggtatcaacagaaaccaggacagccacccaaactcctcatctatcttgcatccaacctagattctggggtccctgccaggttcagtggcagtgggtctgggacagacttcaccctcaacatccatcctgtggaggaggaggatactgcaacctattactgtcagcacagtagggagtttccgctcacgttcggtgctgggaccaagctggagctgaaa

SEQ ID NO: 101 - protein, 15 aa, Mus musculus
RANKSVSASGYSFMH

SEQ ID NO: 102 - protein, 7 aa, Mus musculus
LASNLDS

SEQ ID NO: 103 - protein, 9 aa, Mus musculus
QHSREFPLT

SEQ ID NO: 104 - protein, 120 aa, Mus musculus
QVQLKQSGPGLVQPSQSLSITCTVSGFSLTTYGVHWVRQSPGKGLEWLGVIWSAGITDYNAPFISRLSITKDNSKSQVFFKMNSLQADDTAIYYCARNDYYGNLYAMDYWGQGTSVTVSS

SEQ ID NO: 105 - DNA, 360 bp, Mus musculus
caggtccagctgaagcagtcaggacctggcctagtgcagccctcacagagcctgtccatcacctgcacagtctctggtttctcattaactacctatggtgtacactgggttcgccagtctccaggaaagggtctggagtggctgggagtgatatggagtgctggaatcacagactataatgcacctttcatatccagactgagcatcaccaaggacaattccaagagccaagttttctttaaaatgaacagtctgcaagctgatgacacagccatatattactgtgccagaaatgactactatggtaacctctatgctatggactactggggtcaaggaacctcagtcaccgtctcctca

SEQ ID NO: 106 - protein, 16 aa, Mus musculus
VIWSAGITDYNAPFIS

SEQ ID NO: 107 - protein, 12 aa, Mus musculus
NDYYGNLYAMDY

SEQ ID NO: 108 - protein, 111 aa, Mus musculus
DIVLTQSPASLAVSLGQRATISCRANKSVSASGYTFMHWYQQKPGQPPKLLIYLVSNLASGVPARFSGSGSGTDFTLNIHPVEGEDAATYYCQHSREFPLTFGAGTKLELK

SEQ ID NO: 109 - DNA, 333 bp, Mus musculus
gacattgtgctgacacagtctcctgcttccttagctgtatctctggggcagagggccaccatctcatgcagggccaacaagagtgtcagtgcatctggctatacttttatgcactggtaccaacagaaaccaggacagccacccaagctcctcatctatctagtatccaacctagcatctggggtccctgccaggttcagtggcagtgggtctgggacagacttcaccctcaacatccatcctgtggagggggaggatgctgcaacctattactgtcagcacagtagggagtttccgctcacgttcggtgctgggaccaagctggagctgaaa

SEQ ID NO: 110 - protein, 15 aa, Mus musculus
RANKSVSASGYTFMH

SEQ ID NO: 111 - protein, 7 aa, Mus musculus
LVSNLAS

SEQ ID NO: 112 - protein, 119 aa, Mus musculus
QVQLKQSGPGLVQPSQSLSITCTVSDFSLTIFGVHWVRQSPGKGLEWLGVIWRDGSTDYNAALMSRLNITKDNSKSQVFFKMNSLQTDDTAIYYCAKNRRYDYAWFPYWGQGTLVSVSA

SEQ ID NO: 113 - DNA, 357 bp, Mus musculus
caggtgcaactgaaacagtcaggacctggcctagtgcagccctcacagagcctgtccataacctgcacagtctctgatttctcattaactatctttggggttcactgggttcgccagtctccaggaaagggtctggagtggctgggagtgatttggagagatggaagcacagactataatgcagctctcatgtccagactgaatatcaccaaggacaactccaagagccaagttttctttaaaatgaacagtctgcaaactgatgacactgccatatattactgtgccaaaaatcggaggtatgattacgcctggtttccttattggggccaagggactctggtctctgtctctgca

SEQ ID NO: 114 - protein, 9 aa, Mus musculus
FSLTIFGVH

SEQ ID NO: 115 - protein, 16 aa, Mus musculus
VIWRDGSTDYNAALMS

SEQ ID NO: 116 - protein, 11 aa, Mus musculus
NRRYDYAWFPY

SEQ ID NO: 117 - protein, 111 aa, Mus musculus
DIVLTQSPASLAVSLGQRATISCRASKSVSASGYSFLHWYQQKPGQPPKLLIYLTSNLESGVPARFSGSGSGTDFTLNIHPVEEEDAATYYCQHSRDFPPTFGAGTKLELK

SEQ ID NO: 118 - DNA, 333 bp, Mus musculus
gacattgtgctgacacagtctcctgcttccttagctgtatctctggggcagagggccaccatctcatgcagggccagcaaaagtgtcagtgcatctggctatagttttttgcactggtaccaacagaaaccaggacagccacccaaactcctcatttatcttacatccaacctagaatctggggtccctgccaggttcagtggcagtgggtctgggacagacttcaccctcaacatccatcctgtggaggaggaggatgctgcaacctattactgtcagcacagtagggactttcctcccacgttcggggctgggaccaagctggagctgaaa

SEQ ID NO: 119 - protein, 15 aa, Mus musculus
RASKSVSASGYSFLH

SEQ ID NO: 120 - protein, 7 aa, Mus musculus
LTSNLES

SEQ ID NO: 121 - protein, 9 aa, Mus musculus
QHSRDFPPT

SEQ ID NO: 122 - protein, 120 aa, Mus musculus
QVQLKQSGPGLVQPSQKLSITCTVSGFSLTTYGVHWIRQSPVKGLEWLGVIWTTGVVDYNAAFISRLNITKDNSKSQIFFKMNSLQTNDTAMYYCARNSYYGNLYVMDYWGQGTSVTVSS

SEQ ID NO: 123 - DNA, 360 bp, Mus musculus
caggtgcaactgaaacagtcaggacctggcctagtgcagccctcacagaagttgtccattacctgcacagtctctggtttctcattaactacctatggtgtgcactggattcgccagtctccagtaaagggtctggagtggctgggagtgatatggactactggagttgtagactataatgcagctttcatatccagactgaacatcaccaaggacaattccaagagccaaattttctttaaaatgaacagtctgcaaactaatgacacagccatgtattactgtgccagaaattcctactatggaaacctctatgttatggactactggggtcaaggaacctcagtcaccgtctcctca

SEQ ID NO: 124 - protein, 16 aa, Mus musculus
VIWTTGVVDYNAAFIS

SEQ ID NO: 125 - protein, 111 aa, Mus musculus
DIVLTQSPASLPIFLGQRATISCRASRSVSASGYTFMHWYQQKPGQPPKLLIYLVSNLESGVPARFSGSGSGTDFTLNIHPVEEEDAATYYCQHSREFPLTFGAGTKLELK

SEQ ID NO: 126 - DNA, 333 bp, Mus musculus
gacattgtgctgacacagtctcctgcttccttacctatatttctggggcagagggccaccatctcatgcagggccagcagaagtgtcagtgcatctggctatacttttatgcactggtaccaacagaaaccaggacagccacccaaactcctcatctatcttgtatccaacctagaatctggggtccctgccaggttcagtggcagtgggtctgggacagacttcaccctcaacatccatcctgtggaggaggaggatgctgcaacctattactgtcagcacagtagggagtttcctctcacgttcggtgctgggaccaagctggagctgaaa

SEQ ID NO: 127 - protein, 15 aa, Mus musculus
RASRSVSASGYTFMH

SEQ ID NO: 128 - protein, 7 aa, Mus musculus
LVSNLES

SEQ ID NO: 129 - protein, 119 aa, Mus musculus
QVQLKQSGPGPVQPSQSLSITCTVSDFSLTIFGIHWVRQSPGKGLEWLGVIWRDGSTDYNVALMSRLNITKDNSKSQVFFKMNSLQTDDTAIYYCAKNRRYDYAWFPYWGQGTLVSVSA

SEQ ID NO: 130 - DNA, 357 bp, Mus musculus
caggtgcaactgaaacagtcaggacctggcccagtgcagccctcacagagcctatccataacctgcacagtctctgatttctcattaactatctttgggattcactgggttcgccagtctccaggaaagggtctggagtggctgggagtgatttggagagatggaagcacagactacaatgtagctctcatgtccagactgaacatcaccaaggacaactccaagagtcaagttttctttaaaatgaacagtctacaaactgatgacactgccatatactactgtgccaaaaatcggaggtatgattacgcctggtttccttactggggccaagggactctggtctctgtctctgca

SEQ ID NO: 131 - protein, 9 aa, Mus musculus
FSLTIFGIH

SEQ ID NO: 132 - protein, 16 aa, Mus musculus
VIWRDGSTDYNVALMS

SEQ ID NO: 133 - protein, 119 aa, Homo sapiens
QIQLVQSGSELKKPGASVKVSCKASGYTFTNYGMNWVRQAPGQGLEWMGWINTYTGEPTYADGFTGRFVFSLDTSASTAYLQISSLKAEDTAVYFCAREEDYRYVFNYWGQGTLVTVSS

SEQ ID NO: 134 - DNA, 357 bp, Homo sapiens
cagattcagctggtgcagtctggcagcgagctgaagaaacctggcgcctctgtgaaggtgtcctgcaaggctagcggctacacattcaccaactacggcatgaactgggtccgacaggctcctggacagggactcgaatggatgggctggatcaacacctacaccggcgagcctacctacgccgatggcttcacaggcagattcgtgttcagcctggacaccagcgccagcacagcttacctgcagatcagctctctgaaggccgaggataccgccgtgtacttctgcgccagagaagaggactaccgctacgtgttcaactactggggccagggcacactggtcaccgtttcttct

SEQ ID NO: 135 - protein, 17 aa, Homo sapiens
WINTYTGEPTYADGFTG

SEQ ID NO: 136 - protein, 119 aa, Homo sapiens
QVQLVQSGSELKKPGASVKVSCKASGYTFTNYGMNWVRQAPGQGLEWMGWINTYTGEPTYADGFTGRFVFSLDTSASTAYLQISSLKAEDTAVYFCAREEDYRYVFNYWGQGTLVTVSS

SEQ ID NO: 137 - DNA, 357 bp, Homo sapiens
caggttcagctggtgcagtctggcagcgagctgaagaaacctggcgcctctgtgaaggtgtcctgcaaggctagcggctacacattcaccaactacggcatgaactgggtccgacaggctcctggacagggactcgaatggatgggctggatcaacacctacaccggcgagcctacctacgccgatggcttcacaggcagattcgtgttcagcctggacaccagcgccagcacagcttacctgcagatcagctctctgaaggccgaggataccgccgtgtacttctgcgccagagaagaggactaccgctacgtgttcaactactggggccagggcacactggtcaccgtttcttct

SEQ ID NO: 138 - protein, 119 aa, Homo sapiens
QVQLVQSGSELKKPGASVKVSCKASGYTFTNYGMNWVRQAPGQGLEWMGWINTYTGEPTYADGFTGRFVFSLDTSASTAYLQISSLKAEDTAVYYCAREEDYRYVFNYWGQGTLVTVSS

SEQ ID NO: 139 - DNA, 357 bp, Homo sapiens
caggttcagctggtgcagtctggcagcgagctgaagaaacctggcgcctctgtgaaggtgtcctgcaaggctagcggctacacattcaccaactacggcatgaactgggtccgacaggctcctggacagggactcgaatggatgggctggatcaacacctacaccggcgagcctacctacgccgatggcttcacaggcagattcgtgttcagcctggacaccagcgccagcacagcttacctgcagatcagctctctgaaggccgaggataccgccgtgtactactgcgccagagaagaggactaccgctacgtgttcaactactggggccagggcacactggtcaccgtttcttct

SEQ ID NO: 140 - protein, 120 aa, Homo sapiens
QVQLVQSGAEVKKPGSSVKVSCKASGYTFTDYVIHWVRQAPGQGLEWMGYLHPYNDDTKYNEKFQGRVTLTSDKSSSTAYMELSSLRSEDTAVYYCARRGYYDYAWFADWGQGTLVTVSS

SEQ ID NO: 141 - DNA, 360 bp, Homo sapiens
caggttcagctggttcagtctggcgccgaagtgaagaaacctggcagcagcgtgaaggtgtcctgcaaggctagcggctacacattcaccgactacgtgatccactgggtccgacaggctccaggacagggacttgagtggatgggctatctgcacccctacaacgacgacaccaagtacaacgagaagttccagggcagagtgaccctcaccagcgacaagtctagcagcaccgcctacatggaactgagcagcctgagaagcgaggacaccgccgtgtactactgtgccagaagaggctactacgactacgcttggtttgccgattggggccagggaaccctggtcacagttagctct

SEQ ID NO: 142 - protein, 17 aa, Homo sapiens
YLHPYNDDTKYNEKFQG

SEQ ID NO: 143 - protein, 120 aa, Homo sapiens
QVQLVQSGAEVKKPGSSVKVSCKASGYTFTDYVIHWVRQAPGQGLEWMGYLHPYNDDTKYNEKFQGRVTITADKSSSTAYMELSSLRSEDTAVYYCARRGYYDYAWFADWGQGTLVTVSS

SEQ ID NO: 144 - DNA, 360 bp, Homo sapiens
caggttcagctggttcagtctggcgccgaagtgaagaaacctggcagcagcgtgaaggtgtcctgcaaggctagcggctacacattcaccgactacgtgatccactgggtccgacaggctccaggacagggacttgagtggatgggctatctgcacccctacaacgacgacaccaagtacaacgagaagttccagggcagagtgaccatcaccgccgacaagtctagcagcaccgcctacatggaactgagcagcctgagaagcgaggacaccgccgtgtactactgtgccagaagaggctactacgactacgcttggtttgccgattggggccagggaaccctggtcacagttagctct

SEQ ID NO: 145 - protein, 120 aa, Homo sapiens
QVQLVQSGAEVKKPGSSVKVSCKASGYTFTDYVIHWVRQAPGQGLEWMGYLHPYNDDTKYNEKFQGRVTITADESTSTAYMELSSLRSEDTAVYYCARRGYYDYAWFADWGQGTLVTVSS

SEQ ID NO: 146 - DNA, 360 bp, Homo sapiens
caggttcagctggttcagtctggcgccgaagtgaagaaacctggcagcagcgtgaaggtgtcctgcaaggctagcggctacacattcaccgactacgtgatccactgggtccgacaggctccaggacagggacttgagtggatgggctatctgcacccctacaacgacgacaccaagtacaacgagaagttccagggcagagtgaccatcaccgccgacgagtctaccagcaccgcctacatggaactgagcagcctgagaagcgaggacaccgccgtgtactactgtgccagaagaggctactacgactacgcttggtttgccgattggggccagggaaccctggtcacagttagctct

SEQ ID NO: 147 - protein, 107 aa, Homo sapiens
DIQMTQSPSSLSASVGDRVTITCQASQDISNYLNWYQQKPGKAPKLLIYDTSRLHAGVPSRFSGSGSGTDYTFTISSLQPEDIATYFCQQGVTLPLTFGQGTKLEIK

SEQ ID NO: 148 - DNA, 321 bp, Homo sapiens
gacatccagatgacacagagccctagcagcctgtctgccagcgtgggagacagagtgaccatcacctgtcaggccagccaggacatcagcaactacctgaactggtatcagcagaagcccggcaaggcccctaagctgctgatctacgacaccagcagactgcacgctggcgtgccatctagattcagcggctctggctctggcaccgactacaccttcacaatcagcagcctgcagcctgaggatatcgctacctacttctgccagcaaggcgtgaccctgcctctgacatttggccagggcaccaagctggaaatcaag

SEQ ID NO: 149 - protein, 11 aa, Homo sapiens
QASQDISNYLN

SEQ ID NO: 150 - protein, 107 aa, Homo sapiens
DIQMTQSPSSLSASVGDRVTITCQASQDISNYLNWYQQKPGKAPKLLIYDTSRLHAGVPSRFSGSGSGTDFTFTISSLQPEDIATYFCQQGVTLPLTFGQGTKLEIK

SEQ ID NO: 151 - DNA, 321 bp, Homo sapiens
gacatccagatgacacagagccctagcagcctgtctgccagcgtgggagacagagtgaccatcacctgtcaggccagccaggacatcagcaactacctgaactggtatcagcagaagcccggcaaggcccctaagctgctgatctacgacaccagcagactgcacgctggcgtgccatctagattcagcggctctggctctggcaccgacttcaccttcacaatcagcagcctgcagcctgaggatatcgctacctacttctgccagcaaggcgtgaccctgcctctgacatttggccagggcaccaagctggaaatcaag

SEQ ID NO: 152 - protein, 107 aa, Homo sapiens
DIQMTQSPSSLSASVGDRVTITCQASQDISNYLNWYQQKPGKAPKLLIYDTSRLHAGVPSRFSGSGSGTDFTFTISSLQPEDIATYYCQQGVTLPLTFGQGTKLEIK

SEQ ID NO: 153 - DNA, 321 bp, Homo sapiens
gacatccagatgacacagagccctagcagcctgtctgccagcgtgggagacagagtgaccatcacctgtcaggccagccaggacatcagcaactacctgaactggtatcagcagaagcccggcaaggcccctaagctgctgatctacgacaccagcagactgcacgctggcgtgccatctagattcagcggctctggctctggcaccgacttcaccttcacaatcagcagcctgcagcctgaggatatcgctacctactactgccagcaaggcgtgaccctgcctctgacatttggccagggcaccaagctggaaatcaag

SEQ ID NO: 154 - protein, 111 aa, Homo sapiens
DIVLTQSPASLAVSPGQRATITCRASKSVSASGYTWMHWYQQKPGQPPKLLIYLASNLESGVPARFSGSGSGTDFTLTINPVEANDTANYYCQHSRELPPTFGQGTKLEIK

SEQ ID NO: 155 - DNA, 333 bp, Homo sapiens
gacatcgtgctgacacagagccctgcttctctggctgtgtctcctggccagagagccaccatcacctgtagagccagcaagagcgtgtccgcctctggctacacatggatgcactggtatcagcagaagcccggccagcctcctaagctgctgatctacctggccagcaacctggaaagcggagtgcctgctagattcagcggctctggctctggcaccgacttcaccctgacaatcaaccccgtggaagccaacgacaccgccaactactactgccagcacagcagagagctgcctccaacatttggccagggcaccaagctggaaatcaag

SEQ ID NO: 156 - protein, 111 aa, Homo sapiens
EIVLTQSPGTLSLSPGERATLSCRASKSVSASGYTWMHWYQQKPGQAPRLLIYLASNLESGIPDRFSGSGSGTDFTLTISRLEPEDFAVYYCQHSRELPPTFGQGTKLEIK

SEQ ID NO: 157 - DNA, 333 bp, Homo sapiens
gagatcgtgctgacacagagccctggcacactgtcactgtctccaggcgagagagccacactgagctgtagagccagcaagagcgtgtccgcctctggctacacatggatgcactggtatcagcagaagcccggccaggctcctagactgctgatctacctggccagcaacctggaaagcggcatccccgatagattcagcggctctggctctggcaccgacttcaccctgacaatcagcagactggaacccgaggacttcgccgtgtactactgccagcacagcagagagctgcctccaacatttggccagggcaccaagctggaaatcaag

SEQ ID NO: 158 - protein, 111 aa, Homo sapiens
EIVLTQSPGTLSLSPGERATLSCRASKSVSASGYTWMHWYQQKPGQAPRLLIYLASSLESGIPDRFSGSGSGTDFTLTISRLEPEDFAVYYCQHSRELPPTFGQGTKLEIK

SEQ ID NO: 159 - DNA, 333 bp, Homo sapiens
gagatcgtgctgacacagagccctggcacactgtcactgtctccaggcgagagagccacactgagctgtagagccagcaagagcgtgtccgcctctggctacacatggatgcactggtatcagcagaagcccggccaggctcctagactgctgatctacctggccagcagcctggaaagcggcatccccgatagattcagcggctctggctctggcaccgacttcaccctgacaatcagcagactggaacccgaggacttcgccgtgtactactgccagcacagcagagagctgcctccaacatttggccagggcaccaagctggaaatcaag

SEQ ID NO: 160 - protein, 7 aa, Homo sapiens
LASSLES

SEQ ID NO: 161 - protein, 8 aa, Artificial Sequence
  synthetically generated protein
GSGSGNGS

SEQ ID NO: 162 - protein, 17 aa, Artificial Sequence
  synthetically generated protein
GSGLNDIFEAQKIEWHE